European Patent Application EP 4 292 611 A1, published December 20, 2023. Title: ANTI-CD112R ANTIBODY AND USE THEREOF. Applicant: Shanghai Junshi Biosciences Co., Ltd. Suzhou Junmeng Biosciences Co., Ltd. The sequence listing filed with the application follows.

SEQUENCE LISTING (150 sequences)

SEQ ID NO: 1 - protein, 5 aa, Artificial Sequence
  HCDR1
NYNIH

SEQ ID NO: 2 - protein, 17 aa, Artificial Sequence
  HCDR2
YVYPYNGVPGYNQKFKS

SEQ ID NO: 3 - protein, 9 aa, Artificial Sequence
  HCDR3
ERGRDYFDS

SEQ ID NO: 4 - protein, 11 aa, Artificial Sequence
  LCDR1
RVSANIYSNLV

SEQ ID NO: 5 - protein, 7 aa, Artificial Sequence
  LCDR2
GGTNLAD

SEQ ID NO: 6 - protein, 9 aa, Artificial Sequence
  LCDR3
QHFWSTPYT

SEQ ID NO: 7 - protein, 5 aa, Artificial Sequence
  HCDR1
SHYMY

SEQ ID NO: 8 - protein, 17 aa, Artificial Sequence
  HCDR2
EINPSNGDTKFNEKFKS

SEQ ID NO: 9 - protein, 10 aa, Artificial Sequence
  HCDR3
EKDAFSALDY

SEQ ID NO: 10 - protein, 11 aa, Artificial Sequence
  LCDR1
RASQGIRGHLD

SEQ ID NO: 11 - protein, 7 aa, Artificial Sequence
  LCDR2
STSILNF

SEQ ID NO: 12 - protein, 9 aa, Artificial Sequence
  LCDR3
LQRNAYPLT

SEQ ID NO: 13 - protein, 5 aa, Artificial Sequence
  HCDR1
SYHMS

SEQ ID NO: 14 - protein, 17 aa, Artificial Sequence
  HCDR2
AINSNDINTYYLDTVKG

SEQ ID NO: 15 - protein, 11 aa, Artificial Sequence
  HCDR3
HEDYYGFAMDY

SEQ ID NO: 16 - protein, 5 aa, Artificial Sequence
  HCDR1
DYFIH

SEQ ID NO: 17 - protein, 17 aa, Artificial Sequence
  HCDR2
WIIPASGDTDCAPIFQG

SEQ ID NO: 18 - protein, 10 aa, Artificial Sequence
  HCDR3
WVWSPYAVDY

SEQ ID NO: 19 - protein, 10 aa, Artificial Sequence
  LCDR1
SATSSINYMH

SEQ ID NO: 20 - protein, 7 aa, Artificial Sequence
  LCDR2
DTSKLAS

SEQ ID NO: 21 - protein, 9 aa, Artificial Sequence
  LCDR3
QQWTSNPLT

SEQ ID NO: 22 - protein, 5 aa, Artificial Sequence
  HCDR1
NYIMS

SEQ ID NO: 23 - protein, 17 aa, Artificial Sequence
  HCDR2
TISSGGSSTYYVDRVKG

SEQ ID NO: 24 - protein, 14 aa, Artificial Sequence
  HCDR3
HEDWDPLYYYSMDY

SEQ ID NO: 25 - protein, 10 aa, Artificial Sequence
  LCDR1
SASSSVSYMY

SEQ ID NO: 26 - protein, 7 aa, Artificial Sequence
  LCDR2
DTSHLAF

SEQ ID NO: 27 - protein, 9 aa, Artificial Sequence
  LCDR3
QQWTTYPLT

SEQ ID NO: 28 - protein, 5 aa, Artificial Sequence
  HCDR1
DYFIH

SEQ ID NO: 29 - protein, 17 aa, Artificial Sequence
  HCDR2
WIIPASGDTDCAPIFQG

SEQ ID NO: 30 - protein, 10 aa, Artificial Sequence
  HCDR3
WVWSPYAVDY

SEQ ID NO: 31 - protein, 17 aa, Artificial Sequence
  LCDR1
KSSQSLLNSGNQKNFLA

SEQ ID NO: 32 - protein, 7 aa, Artificial Sequence
  LCDR2
GASTRES

SEQ ID NO: 33 - protein, 9 aa, Artificial Sequence
  LCDR3
QNDHSYPWT

SEQ ID NO: 34 - protein, 5 aa, Artificial Sequence
  HCDR1
DYNMH

SEQ ID NO: 35 - protein, 17 aa, Artificial Sequence
  HCDR2
YIYPYNGGTGHNQNFKS

SEQ ID NO: 36 - protein, 10 aa, Artificial Sequence
  HCDR3
EDFRHEKMDY

SEQ ID NO: 37 - protein, 11 aa, Artificial Sequence
  LCDR1
RTSDNIYVYLS

SEQ ID NO: 38 - protein, 7 aa, Artificial Sequence
  LCDR2
NAKTLTE

SEQ ID NO: 39 - protein, 9 aa, Artificial Sequence
  LCDR3
QHHYGTPYT

SEQ ID NO: 40 - protein, 5 aa, Artificial Sequence
  HCDR1
SYHMS

SEQ ID NO: 41 - protein, 17 aa, Artificial Sequence
  HCDR2
AISRDGDSTYYPDTVKG

SEQ ID NO: 42 - protein, 11 aa, Artificial Sequence
  HCDR3
HEDYFGFAMDS

SEQ ID NO: 43 - protein, 11 aa, Artificial Sequence
  LCDR1
KASQSVTNDVA

SEQ ID NO: 44 - protein, 7 aa, Artificial Sequence
  LCDR2
YVSNHYT

SEQ ID NO: 45 - protein, 9 aa, Artificial Sequence
  LCDR3
QQAYRSPWT

SEQ ID NO: 46 - protein, 16 aa, Artificial Sequence
  LCDR1
RSSQSIVHSNGNTYLH

SEQ ID NO: 47 - protein, 7 aa, Artificial Sequence
  LCDR2
KVSNRFS

SEQ ID NO: 48 - protein, 9 aa, Artificial Sequence
  LCDR3
FQGSHVPWT

SEQ ID NO: 49 - protein, 5 aa, Artificial Sequence
  HCDR1
SYHMS

SEQ ID NO: 50 - protein, 17 aa, Artificial Sequence
  HCDR2
AINSNVISTYYLDTVKG

SEQ ID NO: 51 - protein, 11 aa, Artificial Sequence
  HCDR3
HEDYYGFAMDY

SEQ ID NO: 52 - protein, 11 aa, Artificial Sequence
  LCDR1
KASQSVSNDVA

SEQ ID NO: 53 - protein, 7 aa, Artificial Sequence
  LCDR2
YVSHRFT

SEQ ID NO: 54 - protein, 9 aa, Artificial Sequence
  LCDR3
HQAYRSPWT

SEQ ID NO: 55 - protein, 5 aa, Artificial Sequence
  HCDR1
DYNMN

SEQ ID NO: 56 - protein, 17 aa, Artificial Sequence
  HCDR2
YIYPYNGGAGYNQNFKN

SEQ ID NO: 57 - protein, 11 aa, Artificial Sequence
  HCDR3
ERGMQRDYFDY

SEQ ID NO: 58 - protein, 11 aa, Artificial Sequence
  LCDR1
RTSENIYSNLA

SEQ ID NO: 59 - protein, 7 aa, Artificial Sequence
  LCDR2
AATNLAD

SEQ ID NO: 60 - protein, 9 aa, Artificial Sequence
  LCDR3
QHFWGTPYT

SEQ ID NO: 61 - protein, 5 aa, Artificial Sequence
  HCDR1
DYNIH

SEQ ID NO: 62 - protein, 17 aa, Artificial Sequence
  HCDR2
YNYPYNGGAGYNQNFRS

SEQ ID NO: 63 - protein, 11 aa, Artificial Sequence
  HCDR3
GEEVRRGPFYF

SEQ ID NO: 64 - protein, 11 aa, Artificial Sequence
  LCDR1
RTSENIYSFLV

SEQ ID NO: 65 - protein, 7 aa, Artificial Sequence
  LCDR2
NAKTLAE

SEQ ID NO: 66 - protein, 9 aa, Artificial Sequence
  LCDR3
QHYYGTPYT

SEQ ID NO: 67 - protein, 5 aa, Artificial Sequence
  HCDR1
SYHMS

SEQ ID NO: 68 - protein, 17 aa, Artificial Sequence
  HCDR2
AINSNGINTYYLDTVKG

SEQ ID NO: 69 - protein, 11 aa, Artificial Sequence
  HCDR3
HEDYYGFAMDY

SEQ ID NO: 70 - protein, 11 aa, Artificial Sequence
  LCDR1
KASQSVSNDVA

SEQ ID NO: 71 - protein, 7 aa, Artificial Sequence
  LCDR2
YVSNRFT

SEQ ID NO: 72 - protein, 9 aa, Artificial Sequence
  LCDR3
QQAYRSPWT

SEQ ID NO: 73 - protein, 5 aa, Artificial Sequence
  HCDR1
DYSMH

SEQ ID NO: 74 - protein, 17 aa, Artificial Sequence
  HCDR2
WISTETAQPTYADDFRG

SEQ ID NO: 75 - protein, 10 aa, Artificial Sequence
  HCDR3
TGNYGWYFSV

SEQ ID NO: 76 - protein, 12 aa, Artificial Sequence
  LCDR1
RATSGVSSSYLF

SEQ ID NO: 77 - protein, 7 aa, Artificial Sequence
  LCDR2
STSNLAS

SEQ ID NO: 78 - protein, 9 aa, Artificial Sequence
  LCDR3
QQYSGYPYT

SEQ ID NO: 79 - protein, 5 aa, Artificial Sequence
  HCDR1
DYPMS

SEQ ID NO: 80 - protein, 16 aa, Artificial Sequence
  HCDR2
CIDTDENTYYPDSVKG

SEQ ID NO: 81 - protein, 11 aa, Artificial Sequence
  HCR3
GWDDYAAWFAY

SEQ ID NO: 82 - protein, 10 aa, Artificial Sequence
  LCDR1
RASSSVNYMY

SEQ ID NO: 83 - protein, 7 aa, Artificial Sequence
  LCDR2
HTSNLAP

SEQ ID NO: 84 - protein, 9 aa, Artificial Sequence
  LCDR3
QQFTSSPWT

SEQ ID NO: 85 - protein, 118 aa, Artificial Sequence
  VH
EVQLQQSGPELVKPGASVKISCKASGYPFINYNIHWLRQSRGKSLEWIGYVYPYNGVPGYNQKFKSKATLTADNSFSTAYMEFRSLTSEDSAVYFCARERGRDYFDSWGQGTSLTVSS

SEQ ID NO: 86 - protein, 107 aa, Artificial Sequence
  VL
DIQLTQSPASLSVSVGETVTITCRVSANIYSNLVWYHQRQGKSPQLLVYGGTNLADGVPSRFSGSGSGTQFSLKINSLQSEDFGSYHCQHFWSTPYTFGGGTKLEIK

SEQ ID NO: 87 - protein, 119 aa, Artificial Sequence
  VH
QVQLQQSGAELVKPGASVKLSCKASGYTFTSHYMYWLKQRPGQGLEWIGEINPSNGDTKFNEKFKSKATLTVDKSSSTAYMQLSSLTSEDSAVYYCTREKDAFSALDYWGQGTSVTDSS

SEQ ID NO: 88 - protein, 107 aa, Artificial Sequence
  VL
DIQMIQSPSSMFASLGDRVSLSCRASQGIRGHLDWYQQKPGGTIKLLIYSTSILNFGVPSRFSGSGSGSDYSLTISSLESEDFADYYCLQRNAYPLTFGAGTKLELK

SEQ ID NO: 89 - protein, 120 aa, Artificial Sequence
  VH
DVQLVESGGGLVKLGGSLKLSCVASGFTFSSYHMSWIRQTPEKRLELVAAINSNDINTYYLDTVKGRFTISRDIAKNTLHLQMSSLKSEDTALYYCARHEDYYGFAMDYWGQGTSVTVSS

SEQ ID NO: 90 - protein, 107 aa, Artificial Sequence; identical to SEQ ID NO: 86
  VL

SEQ ID NO: 91 - protein, 119 aa, Artificial Sequence
  VH
EVQLQQSGAELVRSGTSVTLSCTASGFNIRDYFIHWVKQRPEQGLEWIGWIIPASGDTDCAPIFQGKATLTADTFSNTAYLHLNSLTSEDTAVYYCNTWVWSPYAVDYWGQGTSVTVSS

SEQ ID NO: 92 - protein, 106 aa, Artificial Sequence
  VL
QIVLTQSPAIMSVSPGEKVTMTCSATSSINYMHWYQQKSGTSPKRWIYDTSKLASGVPARFSGSGSGTSYSLTISNMEAEDAATYYCQQWTSNPLTFGAGTKLELK

SEQ ID NO: 93 - protein, 123 aa, Artificial Sequence
  VH
EVMLVESGGGLVKPGGSLKLSCAASGFTFSNYIMSWVRQTPDMRLEWVATISSGGSSTYYVDRVKGGFPFSRDSVKYILYVHTSSLRSADTAIYYCAKHEDWDPLYYYSMDYWGQGTSVTVSS

SEQ ID NO: 94 - protein, 106 aa, Artificial Sequence
  VL
QIVLTQSPTVMSASPGDKVTMTCSASSSVSYMYWFQQKPGSSPRLLIYDTSHLAFGVPSRFSGSRSGTSYSLTISRMEAEDTATYYCQQWTTYPLTFGAGTKLELK

SEQ ID NO: 95 - protein, 119 aa, Artificial Sequence; identical to SEQ ID NO: 91
  VH

SEQ ID NO: 96 - protein, 113 aa, Artificial Sequence
  VL
DIVMTQFPSSLSVPVGEKVTMNCKSSQSLLNSGNQKNFLAWYQQKPGQPPKLLIYGASTRESGVPYRFTGSGSGTDFTLTISSVQAEDLAVYYCQNDHSYPWTFGGGTKLEIK

SEQ ID NO: 97 - protein, 119 aa, Artificial Sequence
  VH
EVQLQQSGPELVKPGASVRISCKASGYTFTDYNMHWVKQSHGKSLEWIGYIYPYNGGTGHNQNFKSKATLTVDKSSSTAYMEFRSLTSDDSAVYYCAREDFRHEKMDYWGQGTSVTVSS

SEQ ID NO: 98 - protein, 107 aa, Artificial Sequence
  VL
DIQMTQSPASLSASVGETVTITCRTSDNIYVYLSWYQQKQGKSPQLLVYNAKTLTENVPSRFSGSGSGTQFSLKINSLQPEDFGSYYCQHHYGTPYTFGGGTKLEIK

SEQ ID NO: 99 - protein, 120 aa, Artificial Sequence
  VH
DVKLVESGGGLVKLGGSLKLSCAASGFTFSSYHMSWVRQTPEKRLELVAAISRDGDSTYYPDTVKGRFTISRDDAENTLYLQMSSLKSEDTALYYCSRHEDYFGFAMDSWGQGTSVTVSS

SEQ ID NO: 100 - protein, 107 aa, Artificial Sequence
  VL
SIVMTQTPKFLLVSAGDRVTITCKASQSVTNDVAWYQQKPGQSPKLLMYYVSNHYTGVPDRFIGSGYGTDFTFTISTVQAEDLAVYFCQQAYRSPWTFGGGTKLEIK

SEQ ID NO: 101 - protein, 119 aa, Artificial Sequence; identical to SEQ ID NO: 91
  VH

SEQ ID NO: 102 - protein, 112 aa, Artificial Sequence
  VL
DVLMTQTPLSLPVSLGDQTSISCRSSQSIVHSNGNTYLHWYLQKPGQSPKLLIYKVSNRFSGVPDRFSGSGSGTDFTLKISRVEAEDLGVYYCFQGSHVPWTFGGGTRLEIK

SEQ ID NO: 103 - protein, 120 aa, Artificial Sequence
  VH
DVKLVESGGGLVKLGGSLKLSCAASGFTFSSYHMSWVRQTPEKRLELVAAINSNVISTYYLDTVKGRFTISRDNAKNTLYLQMSSLKSEDTALYYCARHEDYYGFAMDYWGQGTSVTVSS

SEQ ID NO: 104 - protein, 107 aa, Artificial Sequence
  VL
SIVMTQTPKFLLVSAGDRVTITCKASQSVSNDVAWYQEKPGQSPKLLMYYVSHRFTGVPDRFTGSGYGTDFTFTINTVQAEDLAVYFCHQAYRSPWTFGGGTKLEIK

SEQ ID NO: 105 - protein, 120 aa, Artificial Sequence
  VH
EVQLQQSGPELVRPGASVRISCKASGYTFTDYNMNWVKQSHGKSLEWIGYIYPYNGGAGYNQNFKNKATLTVDTYSRAAYMELRSLTSEDSAVYYCARERGMQRDYFDYWGQGTILTVSS

SEQ ID NO: 106 - protein, 107 aa, Artificial Sequence
  VL
DIQMTQSPASLSVSVGETVTITCRTSENIYSNLAWYQQKQGKSPQLLVYAATNLADGVPSRFSGSGSGTQFSLKINSLQSGDFGSYFCQHFWGTPYTFGGGTKLEIK

SEQ ID NO: 107 - protein, 119 aa, Artificial Sequence
  VH
EVQLQQSGPELVKPGASVKISCKASGYTFTDYNIHWVKQSHGKRPDWIGYNYPYNGGAGYNQNFRSRATLTVDKFSSTAYMELRSLTSEDSAVYYCAGEEVRRGPFYFWGQGTSVTVSS

SEQ ID NO: 108 - protein, 107 aa, Artificial Sequence
  VL
DIQMTQSPDSLSASVGETVTITCRTSENIYSFLVWYQQKQGKSPQLLVYNAKTLAEGVPSRFSGSGSGTQFSLKINSLQPEDFGTYYCQHYYGTPYTFGGGTKLEIK

SEQ ID NO: 109 - protein, 120 aa, Artificial Sequence
  VH
DVKLVESGGGLVKLGGSLKLSCAASGFTFSSYHMSWIRQTPEKRLELVAAINSNGINTYYLDTVKGRFTISRDNAKNTLYLQMSSLKSEDTALYYCARHEDYYGFAMDYWGQGTSVTVSS

SEQ ID NO: 110 - protein, 107 aa, Artificial Sequence
  VL
SIVMTQTPKFLLVSAGDRVTITCKASQSVSNDVAWYQQKPGQSPKLLMYYVSNRFTGVPDRFTGSGYGTDFTFTINTVQAEDLAVYFCQQAYRSPWTFGGGTKLEIK

SEQ ID NO: 111 - protein, 118 aa, Artificial Sequence
  VH
QIQLVQSGPELKKPGETVKISCKASGYTFTDYSMHWVKQAPGKGLKWVGWISTETAQPTYADDFRGRFAFSLETSASTAYLQINNLRNEDTATYFCATGNYGWYFSVWGAGTTVTVSS

SEQ ID NO: 112 - protein, 108 aa, Artificial Sequence
  VL
ENVLTQSPAIMSASPGEKVTMTCRATSGVSSSYLFWYQQKSGASPKIWIYSTSNLASGVPTRFSGSGSGTSYSLTISSVEAEDAATYYCQQYSGYPYTFGGGTKLEIK

SEQ ID NO: 113 - protein, 119 aa, Artificial Sequence
  VH
EVKLVESGGGLVKPGGSLKVSCAASGFTFSDYPMSWVRQTPDKRLEWVACIDTDENTYYPDSVKGRFTISRDNGRNIVNLQMSSLRSEDAAMYYCARGWDDYAAWFAYWGQGTLVTVSA

SEQ ID NO: 114 - protein, 106 aa, Artificial Sequence
  VL
ENVLTQFPAIMSVFLGERVTMSCRASSSVNYMYWYQQKSDASPKLWIYHTSNLAPGVPARFSGSGSGNSYSLTISSMEGEDAATYYCQQFTSSPWTFGGGTKLEIK

SEQ ID NO: 115 - protein, 120 aa, Artificial Sequence
  VH
EVQLVESGGGLVQPGGSLRLSCAASGFTFSSYHMSWVRQAPGKGLELVAAINSNDINTYYLDTVKGRFTISRDIAKNSLYLQMNSLRAEDTAVYYCARHEDYYGFAMDYWGQGTLVTVSS

SEQ ID NO: 116 - protein, 120 aa, Artificial Sequence
  VH
EVQLVESGGGLVKPGGSLRLSCAASGFTFSSYHMSWVRQAPGKGLELVSAINSNDINTYYLDTVKGRFTISRDIAKNSLYLQMNSLRAEDTAVYYCARHEDYYGFAMDYWGQGTLVTVSS

SEQ ID NO: 117 - protein, 120 aa, Artificial Sequence
  VH
EVQLVESGGGLVKPGGSLRLSCAASGFTFSSYHMSWIRQAPGKGLELVSAINSNDINTYYLDTVKGRFTISRDNAKNSLYLQMNSLRAEDTAVYYCARHEDYYGFAMDYWGQGTLVTVSS

SEQ ID NO: 118 - protein, 120 aa, Artificial Sequence
  VH
EVQLVESGGGLVKPGGSLRLSCAASGFTFSSYHMSWVRQAPGKGLELVSAISRDGDSTYYPDTVKGRFTISRDNAKNSLYLQMNSLRAEDTAVYYCSRHEDYFGFAMDSWGQGTLVTVSS

SEQ ID NO: 119 - protein, 120 aa, Artificial Sequence
  VH
EVQLVESGGGLVKPGGSLRLSCAASGFTFSSYHMSWVRQAPGKGLELVSAISRDGDSTYYPDTVKGRFTISRDDAENSLYLQMNSLRAEDTAVYYCSRHEDYFGFAMDSWGQGTLVTVSS

SEQ ID NO: 120 - protein, 120 aa, Artificial Sequence
  VH
EVQLVESGGGLVQPGGSLRLSCAASGFTFSSYHMSWVRQAPGKGLELVAAISRDGDSTYYPDTVKGRFTISRDNAKNSLYLQMNSLRAEDTAVYYCSRHEDYFGFAMDSWGQGTLVTVSS

SEQ ID NO: 121 - protein, 120 aa, Artificial Sequence
  VH
EVQLVESGGGLVQPGGSLRLSCAASGFTFSSYHMSWVRQAPGKGLELVAAISRDGDSTYYPDTVKGRFTISRDDAENSLYLQMNSLRAEDTAVYYCSRHEDYFGFAMDSWGQGTLVTVSS

SEQ ID NO: 122 - protein, 107 aa, Artificial Sequence
  VL
DIVMTQSPDSLAVSLGERATINCKASQSVTNDVAWYQQKPGQPPKLLIYYVSNHYTGVPDRFSGSGSGTDFTLTISSLQAEDVAVYFCQQAYRSPWTFGQGTKLEIK

SEQ ID NO: 123 - protein, 107 aa, Artificial Sequence
  VL
AIQMTQSPSSLSASVGDRVTITCKASQSVTNDVAWYQQKPGKAPKLLIYYVSNHYTGVPSRFSGSGSGTDFTLTISSLQPEDFATYFCQQAYRSPWTFGQGTKLEIK

SEQ ID NO: 124 - protein, 120 aa, Artificial Sequence
  VH
EVQLVESGGGLVQPGGSLRLSCAASGFTFSSYHMSWVRQAPGKGLELVSAINSNVISTYYLDTVKGRFTISRDNAKNSLYLQMNSLRAEDTAVYYCARHEDYYGFAMDYWGQGTLVTVSS

SEQ ID NO: 125 - protein, 120 aa, Artificial Sequence
  VH
EVQLVESGGGLVKPGGSLRLSCAASGFTFSSYHMSWVRQAPGKGLELVSAINSNVISTYYLDTVKGRFTISRDNAKNSLYLQMNSLRAEDTAVYYCARHEDYYGFAMDYWGQGTLVTVSS

SEQ ID NO: 126 - protein, 107 aa, Artificial Sequence
  VL
EIVMTQSPPTLSLSPGERVTLSCKASQSVSNDVAWYQEKPGQAPRLLIYYVSHRFTGIPARFSGSGSGTDFTLTISSLQPEDFAVYYCHQAYRSPWTFGQGTKLEIK

SEQ ID NO: 127 - protein, 107 aa, Artificial Sequence
  VL
DIVMTQSPDSLAVSLGERATINCKASQSVSNDVAWYQQKPGQPPKLLIYYVSHRFTGVPDRFSGSGSGTDFTLTISSLQAEDVAVYFCHQAYRSPWTFGQGTKLEIK

SEQ ID NO: 128 - protein, 120 aa, Artificial Sequence
  VH
EVQLVESGGGLVKPGGSLRLSCAASGFTFSSYHMSWVRQAPGKGLELVSAINSNGINTYYLDTVKGRFTISRDNAKNSLYLQMNSLRAEDTAVYYCARHEDYYGFAMDYWGQGTLVTVSS

SEQ ID NO: 129 - protein, 120 aa, Artificial Sequence
  VH
EVQLVESGGGLVQPGGSLRLSCAASGFTFSSYHMSWIRQAPGKGLELVAAINSNGINTYYLDTVKGRFTISRDNAKNSLYLQMNSLRAEDTAVYYCARHEDYYGFAMDYWGQGTLVTVSS

SEQ ID NO: 130 - protein, 120 aa, Artificial Sequence
  VH
EVQLVESGGGLVQPGGSLRLSCAASGFTFSSYHMSWIRQAPGKGLELVAAINSNDINTYYLDTVKGRFTISRDNAKNSLYLQMNSLRAEDTAVYYCARHEDYYGFAMDYWGQGTLVTVSS

SEQ ID NO: 131 - protein, 107 aa, Artificial Sequence
  VL
DIQMTQSPSSLSASVGDRVTITCKASQSVSNDVAWYQQKPGKAPKLLIYYVSNRFTGVPSRFSGSGSGTDFTLTISSLQPEDFATYFCQQAYRSPWTFGQGTKLEIK

SEQ ID NO: 132 - protein, 107 aa, Artificial Sequence
  VL
EIVMTQSPPTLSLSPGERVTLSCKASQSVSNDVAWYQQKPGQAPRLLIYYVSNRFTGIPARFSGSGSGTDFTLTISSLQPEDFAVYFCQQAYRSPWTFGQGTKLEIK

SEQ ID NO: 133 - protein, 214 aa, Artificial Sequence
  LC
DIVMTQSPDSLAVSLGERATINCKASQSVSNDVAWYQQKPGQPPKLLIYYVSHRFTGVPDRFSGSGSGTDFTLTISSLQAEDVAVYFCHQAYRSPWTFGQGTKLEIKRTVAAPSVFIFPPSDEQLKSGTASVVCLLNNFYPREAKVQWKVDNALQSGNSQESVTEQDSKDSTYSLSSTLTLSKADYEKHKVYACEVTHQGLSSPVTKSFNRGEC

SEQ ID NO: 134 - protein, 447 aa, Artificial Sequence
  HC
EVQLVESGGGLVKPGGSLRLSCAASGFTFSSYHMSWVRQAPGKGLELVSAISRDGDSTYYPDTVKGRFTISRDNAKNSLYLQMNSLRAEDTAVYYCSRHEDYFGFAMDSWGQGTLVTVSSASTKGPSVFPLAPCSRSTSESTAALGCLVKDYFPEPVTVSWNSGALTSGVHTFPAVLQSSGLYSLSSVVTVPSSSLGTKTYTCNVDHKPSNTKVDKRVESKYGPPCPPCPAPEFLGGPSVFLFPPKPKDTLMISRTPEVTCVVVDVSQEDPEVQFNWYVDGVEVHNAKTKPREEQFNSTYRVVSVLTVLHQDWLNGKEYKCKVSNKGLPSSIEKTISKAKGQPREPQVYTLPPSQEEMTKNQVSLTCLVKGFYPSDIAVEWESNGQPENNYKTTPPVLDSDGSFFLYSRLTVDKSRWQEGNVFSCSVMHEALHNHYTQKSLSLSLGK

SEQ ID NO: 135 - protein, 450 aa, Artificial Sequence
  HC
EVQLVESGGGLVKPGGSLRLSCAASGFTFSSYHMSWVRQAPGKGLELVSAISRDGDSTYYPDTVKGRFTISRDNAKNSLYLQMNSLRAEDTAVYYCSRHEDYFGFAMDSWGQGTLVTVSSASTKGPSVFPLAPSSKSTSGGTAALGCLVKDYFPEPVTVSWNSGALTSGVHTFPAVLQSSGLYSLSSVVTVPSSSLGTQTYICNVNHKPSNTKVDKKVEPKSCDKTHTCPPCPAPELLGGPSVFLFPPKPKDTLMISRTPEVTCVVVDVSHEDPEVKFNWYVDGVEVHNAKTKPREEQYNSTYRVVSVLTVLHQDWLNGKEYKCKVSNKALPAPIEKTISKAKGQPREPQVYTLPPSRDELTKNQVSLTCLVKGFYPSDIAVEWESNGQPENNYKTTPPVLDSDGSFFLYSKLTVDKSRWQQGNVFSCSVMHEALHNHYTQKSLSLSPGK

SEQ ID NO: 136 - protein, 214 aa, Artificial Sequence; identical to SEQ ID NO: 133
  LC

SEQ ID NO: 137 - protein, 447 aa, Artificial Sequence
  HC
EVQLVESGGGLVKPGGSLRLSCAASGFTFSSYHMSWVRQAPGKGLELVSAINSNGINTYYLDTVKGRFTISRDNAKNSLYLQMNSLRAEDTAVYYCARHEDYYGFAMDYWGQGTLVTVSSASTKGPSVFPLAPCSRSTSESTAALGCLVKDYFPEPVTVSWNSGALTSGVHTFPAVLQSSGLYSLSSVVTVPSSSLGTKTYTCNVDHKPSNTKVDKRVESKYGPPCPPCPAPEFLGGPSVFLFPPKPKDTLMISRTPEVTCVVVDVSQEDPEVQFNWYVDGVEVHNAKTKPREEQFNSTYRVVSVLTVLHQDWLNGKEYKCKVSNKGLPSSIEKTISKAKGQPREPQVYTLPPSQEEMTKNQVSLTCLVKGFYPSDIAVEWESNGQPENNYKTTPPVLDSDGSFFLYSRLTVDKSRWQEGNVFSCSVMHEALHNHYTQKSLSLSLGK

SEQ ID NO: 138 - protein, 450 aa, Artificial Sequence
  HC
EVQLVESGGGLVKPGGSLRLSCAASGFTFSSYHMSWVRQAPGKGLELVSAINSNGINTYYLDTVKGRFTISRDNAKNSLYLQMNSLRAEDTAVYYCARHEDYYGFAMDYWGQGTLVTVSSASTKGPSVFPLAPSSKSTSGGTAALGCLVKDYFPEPVTVSWNSGALTSGVHTFPAVLQSSGLYSLSSVVTVPSSSLGTQTYICNVNHKPSNTKVDKKVEPKSCDKTHTCPPCPAPELLGGPSVFLFPPKPKDTLMISRTPEVTCVVVDVSHEDPEVKFNWYVDGVEVHNAKTKPREEQYNSTYRVVSVLTVLHQDWLNGKEYKCKVSNKALPAPIEKTISKAKGQPREPQVYTLPPSRDELTKNQVSLTCLVKGFYPSDIAVEWESNGQPENNYKTTPPVLDSDGSFFLYSKLTVDKSRWQQGNVFSCSVMHEALHNHYTQKSLSLSPGK

SEQ ID NO: 139 - protein, 214 aa, Artificial Sequence
  LC
DIQMTQSPSSLSASVGDRVTITCKASQSVSNDVAWYQQKPGKAPKLLIYYVSNRFTGVPSRFSGSGSGTDFTLTISSLQPEDFATYFCQQAYRSPWTFGQGTKLEIKRTVAAPSVFIFPPSDEQLKSGTASVVCLLNNFYPREAKVQWKVDNALQSGNSQESVTEQDSKDSTYSLSSTLTLSKADYEKHKVYACEVTHQGLSSPVTKSFNRGEC

SEQ ID NO: 140 - protein, 447 aa, Artificial Sequence
  HC
EVQLVESGGGLVQPGGSLRLSCAASGFTFSSYHMSWIRQAPGKGLELVAAINSNGINTYYLDTVKGRFTISRDNAKNSLYLQMNSLRAEDTAVYYCARHEDYYGFAMDYWGQGTLVTVSSASTKGPSVFPLAPCSRSTSESTAALGCLVKDYFPEPVTVSWNSGALTSGVHTFPAVLQSSGLYSLSSVVTVPSSSLGTKTYTCNVDHKPSNTKVDKRVESKYGPPCPPCPAPEFLGGPSVFLFPPKPKDTLMISRTPEVTCVVVDVSQEDPEVQFNWYVDGVEVHNAKTKPREEQFNSTYRVVSVLTVLHQDWLNGKEYKCKVSNKGLPSSIEKTISKAKGQPREPQVYTLPPSQEEMTKNQVSLTCLVKGFYPSDIAVEWESNGQPENNYKTTPPVLDSDGSFFLYSRLTVDKSRWQEGNVFSCSVMHEALHNHYTQKSLSLSLGK

SEQ ID NO: 141 - protein, 450 aa, Artificial Sequence
  HC
EVQLVESGGGLVQPGGSLRLSCAASGFTFSSYHMSWIRQAPGKGLELVAAINSNGINTYYLDTVKGRFTISRDNAKNSLYLQMNSLRAEDTAVYYCARHEDYYGFAMDYWGQGTLVTVSSASTKGPSVFPLAPSSKSTSGGTAALGCLVKDYFPEPVTVSWNSGALTSGVHTFPAVLQSSGLYSLSSVVTVPSSSLGTQTYICNVNHKPSNTKVDKKVEPKSCDKTHTCPPCPAPELLGGPSVFLFPPKPKDTLMISRTPEVTCVVVDVSHEDPEVKFNWYVDGVEVHNAKTKPREEQYNSTYRVVSVLTVLHQDWLNGKEYKCKVSNKALPAPIEKTISKAKGQPREPQVYTLPPSRDELTKNQVSLTCLVKGFYPSDIAVEWESNGQPENNYKTTPPVLDSDGSFFLYSKLTVDKSRWQQGNVFSCSVMHEALHNHYTQKSLSLSPGK

SEQ ID NO: 142 - protein, 121 aa, Artificial Sequence
  VH
EVQLQQSGAELVKPGASVKISCKASGYTFTDYNMDWVKQSHGKSLEWIGDIHPKYDRTSYNQNFKGKATLTVDKSSRTAYMELRSLTSEDTAVYFCVRINDFDEGFAMDYWGQGTSVTVSS

SEQ ID NO: 143 - protein, 5 aa, Artificial Sequence
  HCDR1
DYNMD

SEQ ID NO: 144 - protein, 17 aa, Artificial Sequence
  HCDR2
DIHPKYDRTSYNQNFKG

SEQ ID NO: 145 - protein, 12 aa, Artificial Sequence
  HCDR3
INDFDEGFAMDY

SEQ ID NO: 146 - protein, 17 aa, Artificial Sequence
  HCDR2
  MUTAGEN (3)..(3): Xaa is N or S
  MUTAGEN (4)..(4): Xaa is S or R
  MUTAGEN (5)..(5): Xaa is N or D
  MUTAGEN (6)..(6): Xaa is D or G or V
  MUTAGEN (7)..(7): Xaa is I or D
  MUTAGEN (8)..(8): Xaa is N or S
  MUTAGEN (12)..(12): Xaa is L or P
AIXXXXXXTYYXDTVKG

SEQ ID NO: 147 - protein, 11 aa, Artificial Sequence
  HCDR3
  MUTAGEN (5)..(5): Xaa is Y or F
  MUTAGEN (11)..(11): Xaa is Y or S
HEDYXGFAMDX

SEQ ID NO: 148 - protein, 11 aa, Artificial Sequence
  LCDR1
  MUTAGEN (7)..(7): Xaa is T or S
KASQSVXNDVA

SEQ ID NO: 149 - protein, 7 aa, Artificial Sequence
  LCDR2
  MUTAGEN (4)..(4): Xaa is N or H
  MUTAGEN (5)..(5): Xaa is H or R
  MUTAGEN (6)..(6): Xaa is Y or F
YVSXXXT

SEQ ID NO: 150 - protein, 9 aa, Artificial Sequence
  LCDR3
  MUTAGEN (1)..(1): Xaa is Q or H
XQAYRSPWT